European Patent Application EP 4 692 359 A1, published February 11, 2026. Title: Method for production of virus. Applicant: FUJIFILM Corporation. The sequence listing filed with the application follows.

SEQUENCE LISTING (3 sequences)

SEQ ID NO: 1 - DNA, 6073 bp, synthetic construct
  misc_feature 1..6073: note = plasmid
  source 1..6073: mol_type = other DNA
gatccacgggtggcatccctgtgacccctccccagtgcctctcctggccctggaagttgccactccagtgcccaccagccttgtcctaataaaattaagttgcatcattttgtctgactaggtgtccttctataatattatggggtggaggggggtggtatggagcaaggggcaagttgggaagacaacctgtagggcctgcggggtctattgggaaccaagctggagtgcagtggcacaatcttggctcactgcaatctccgcctcctgggttcaagcgattctcctgcctcagcctcccgagttgttgggattccaggcatgcatgaccaggctcagctaatttttgtttttttggtagagacggggtttcaccatattggccaggctggtctccaactcctaatctcaggtgatctacccaccttggcctcccaaattgctgggattacaggcgtgaaccactgctcccttccctgtccttatcgatagatctaggaacccctagtgatggagttggccactccctctctgcgcgctcgctcgctcactgaggccgggcgaccaaaggtcgcccgacgcccgggctttgcccgggcggcctcagtgagcgagcgagcgcgcagctgcctgcaggcagcttggcactggccgtcgttttacaacgtcgtgactgggaaaaccctggcgttacccaacttaatcgccttgcagcacatccccctttcgccagctggcgtaatagcgaagaggcccgcaccgatcgcccttcccaacagttgcgcagcctgaatggcgaatggcgcctgatgcggtattttctccttacgcatctgtgcggtatttcacaccgcatacgtcaaagcaaccatagtacgcgccctgtagcggcgcattaagcgcggcgggtgtggtggttacgcgcagcgtgaccgctacacttgccagcgccctagcgcccgctcctttcgctttcttcccttcctttctcgccacgttcgccggctttccccgtcaagctctaaatcgggggctccctttagggttccgatttagtgctttacggcacctcgaccccaaaaaacttgatttgggtgatggttcacgtagtgggccatcgccctgatagacggtttttcgccctttgacgttggagtccacgttctttaatagtggactcttgttccaaactggaacaacactcaaccctatctcgggctattcttttgatttataagggattttgccgatttcggcctattggttaaaaaatgagctgatttaacaaaaatttaacgcgaattttaacaaaatattaacgtttacaattttatggtgcactctcagtacaatctgctctgatgccgcatagttaagccagccccgacacccgccaacacccgctgacgcgccctgacgggcttgtctgctcccggcatccgcttacagacaagctgtgaccgtctccgggagctgcatgtgtcagaggttttcaccgtcatcaccgaaacgcgcgagacgaaagggcctcgtgatacgcctatttttataggttaatgtcatgataataatggtttcttagacgtcaggtggcacttttcggggaaatgtgcgcggaacccctatttgtttatttttctaaatacattcaaatatgtatccgctcatgagacaataaccctgataaatgcttcaataatattgaaaaaggaagagtatgagtattcaacatttccgtgtcgcccttattcccttttttgcggcattttgccttcctgtttttgctcacccagaaacgctggtgaaagtaaaagatgctgaagatcagttgggtgcacgagtgggttacatcgaactggatctcaacagcggtaagatccttgagagttttcgccccgaagaacgttttccaatgatgagcacttttaaagttctgctatgtggcgcggtattatcccgtattgacgccgggcaagagcaactcggtcgccgcatacactattctcagaatgacttggttgagtactcaccagtcacagaaaagcatcttacggatggcatgacagtaagagaattatgcagtgctgccataaccatgagtgataacactgcggccaacttacttctgacaacgatcggaggaccgaaggagctaaccgcttttttgcacaacatgggggatcatgtaactcgccttgatcgttgggaaccggagctgaatgaagccataccaaacgacgagcgtgacaccacgatgcctgtagcaatggcaacaacgttgcgcaaactattaactggcgaactacttactctagcttcccggcaacaattaatagactggatggaggcggataaagttgcaggaccacttctgcgctcggcccttccggctggctggtttattgctgataaatctggagccggtgagcgtgggtctcgcggtatcattgcagcactggggccagatggtaagccctcccgtatcgtagttatctacacgacggggagtcaggcaactatggatgaacgaaatagacagatcgctgagataggtgcctcactgattaagcattggtaactgtcagaccaagtttactcatatatactttagattgatttaaaacttcatttttaatttaaaaggatctaggtgaagatcctttttgataatctcatgaccaaaatcccttaacgtgagttttcgttccactgagcgtcagaccccgtagaaaagatcaaaggatcttcttgagatcctttttttctgcgcgtaatctgctgcttgcaaacaaaaaaaccaccgctaccagcggtggtttgtttgccggatcaagagctaccaactctttttccgaaggtaactggcttcagcagagcgcagataccaaatactgttcttctagtgtagccgtagttaggccaccacttcaagaactctgtagcaccgcctacatacctcgctctgctaatcctgttaccagtggctgctgccagtggcgataagtcgtgtcttaccgggttggactcaagacgatagttaccggataaggcgcagcggtcgggctgaacggggggttcgtgcacacagcccagcttggagcgaacgacctacaccgaactgagatacctacagcgtgagctatgagaaagcgccacgcttcccgaagggagaaaggcggacaggtatccggtaagcggcagggtcggaacaggagagcgcacgagggagcttccagggggaaacgcctggtatctttatagtcctgtcgggtttcgccacctctgacttgagcgtcgatttttgtgatgctcgtcaggggggcggagcctatggaaaaacgccagcaacgcggcctttttacggttcctggccttttgctggccttttgctcacatgttctttcctgcgttatcccctgattctgtggataaccgtattaccgcctttgagtgagctgataccgctcgccgcagccgaacgaccgagcgcagcgagtcagtgagcgaggaagcggaagagcgcccaatacgcaaaccgcctctccccgcgcgttggccgattcattaatgcagctggcacgacaggtttcccgactggaaagcgggcagtgagcgcaacgcaattaatgtgagttagctcactcattaggcaccccaggctttacactttatgcttccggctcgtatgttgtgtggaattgtgagcggataacaatttcacacaggaaacagctatgaccatgattacgaattgcctgcaggcagctgcgcgctcgctcgctcactgaggccgcccgggcaaagcccgggcgtcgggcgacctttggtcgcccggcctcagtgagcgagcgagcgcgcagagagggagtggccaactccatcactaggggttcctatcgatatcaagctttaatagtaatcaattacggggtcattagttcatagcccatatatggagttccgcgttacataacttacggtaaatggcccgcctggctgaccgcccaacgacccccgcccattgacgtcaataatgacgtatgttcccatagtaacgccaatagggactttccattgacgtcaatgggtggagtatttacggtaaactgcccacttggcagtacatcaagtgtatcatatgccaagtacgccccctattgacgtcaatgacggtaaatggcccgcctggcattatgcccagtacatgaccttatgggactttcctacttggcagtacatctacgtattagtcatcgctattaccatggtgatgcggttttggcagtacatcaatgggcgtggatagcggtttgactcacggggatttccaagtctccaccccattgacgtcaatgggagtttgttttggcaccaaaatcaacgggactttccaaaatgtcgtaacaactccgccccattgacgcaaatgggcggtaggcgtgtacggtgggaggtctatataagcagagctggtttagtggatatccttaagggcccagccggcctcgcgagaattctctagcaagctgtgaccggcgcctacgctagacgccaccatggagagcgacgagagcggcctgcccgccatggagatcgagtgccgcatcaccggcaccctgaacggcgtggagttcgagctggtgggcggcggagagggcacccccaagcagggccgcatgaccaacaagatgaagagcaccaaaggcgccctgaccttcagcccctacctgctgagccacgtgatgggctacggcttctaccacttcggcacctaccccagcggctacgagaaccccttcctgcacgccatcaacaacggcggctacaccaacacccgcatcgagaagtacgaggacggcggcgtgctgcacgtgagcttcagctaccgctacgaggccggccgcgtgatcggcgacttcaaggtggtgggcaccggcttccccgaggacagcgtgatcttcaccgacaagatcatccgcagcaacgccaccgtggagcacctgcaccccatgggcgataacgtgctggtgggcagcttcgcccgcaccttcagcctgcgcgacggcggctactacagcttcgtggtggacagccacatgcacttcaagagcgccatccaccccagcatcctgcagaacgggggccccatgttcgccttccgccgcgtggaggagctgcacagcaacaccgagctgggcatcgtggagtaccagcacgccttcaagacccccatcgccttcgccagatcccgcgctcagtcgtccaattctgccgtggacggcaccgccggacccggctccaccggatctcgcgagggcagaggaagtcttctaacatgcggtgacgtggaggagaatcccggccctatgaccgagtacaagcccacggtgcgcctcgccacccgcgacgacgtccccagggccgtacgcaccctcgccgccgcgttcgccgactaccccgccacgcgccacaccgtcgatccggaccgccacatcgagcgggtcaccgagctgcaagaactcttcctcacgcgcgtcgggctcgacatcggcaaggtgtgggtcgcggacgacggcgccgcggtggcggtctggaccacgccggagagcgtcgaagcgggggcggtgttcgccgagatcggcccgcgcatggccgagttgagcggttcccggctggccgcgcagcaacagatggaaggcctcctggcgccgcaccggcccaaggagcccgcgtggttcctggccaccgtcggcgtctcgcccgaccaccagggcaagggtctgggcagcgccgtcgtgctccccggagtggaggcggccgagcgcgccggggtgcccgccttcctggagacctccgcgccccgcaacctccccttctacgagcggctcggcttcaccgtcaccgccgacgtcgaggtgcccgaaggaccgcgcacctggtgcatgacccgcaagcccggtgcctgaaatcaacctctggattacaaaatttgtgaaagattgactggtattcttaactatgttgctccttttacgctatgtggatacgctgctttaatgcctttgtatcagtt

SEQ ID NO: 2 - DNA, 11920 bp, synthetic construct
  misc_feature 1..11920: note = plasmid
  source 1..11920: mol_type = other DNA
atgactctcttaaggtagccaaatttccataggctccgcccccctgacgagcatcacaaaaatcgacgctcaagtcagaggtggcgaaacccgacaggactataaagataccaggcgtttccccctggaagctccctcgtgcgctctcctgttccgaccctgccgcttaccggatacctgtccgcctttctcccttcgggaagcgtggcgctttctcatagctcacgctgtaggtatctcagttcggtgtaggtcgttcgctccaagctgggctgtgtgcacgaaccccccgttcagcccgaccgctgcgccttatccggtaactatcgtcttgagtccaacccggtaagacacgacttatcgccactggcagcagccactggtaacaggattagcagagcgaggtatgtaggcggtgctacagagttcttgaagtggtggcctaactacggctacactagaaggacagtatttggtatctgcgctctgctgaagccagttaccttcggaaaaagagttggtagctcttgatccggcaaacaaaccaccgctggtagcggtggtttttttgtttgcaagcagcagattacgcgcagaaaaaaaggatctcaagaagatcctttgatcttttctacggggtctgacgctcagtggaacgaaaactcacgttaagggattttggtcatgagattatcaaaaaggatcttcacctagatccttttaaattaaaaatgaagttttaaatcaatctaaagtatatatgagtaaacttggtctgacagttaccaatgcttaatcagtgaggcacctatctcagcgatctgtctatttcgttcatccatagttgcctgactccccgtcgtgtagataactacgatacgggagggcttaccatctggccccagtgctgcaatgataccgcgagacccacgctcaccggctccagatttatcagcaataaaccagccagccggaagggccgagcgcagaagtggtcctgcaactttatccgcctccatccagtctattaattgttgccgggaagctagagtaagtagttcgccagttaatagtttgcgcaacgttgttgccattgctacaggcatcgtggtgtcacgctcgtcgtttggtatggcttcattcagctccggttcccaacgatcaaggcgagttacatgatcccccatgttgtgcaaaaaagcggttagctccttcggtcctccgatcgttgtcagaagtaagttggccgcagtgttatcactcatggttatggcagcactgcataattctcttactgtcatgccatccgtaagatgcttttctgtgactggtgagtactcaaccaagtcattctgagaatagtgtatgcggcgaccgagttgctcttgcccggcgtcaatacgggataataccgcgccacatagcagaactttaaaagtgctcatcattggaaaacgttcttcggggcgaaaactctcaaggatcttaccgctgttgagatccagttcgatgtaacccactcgtgcacccaactgatcttcagcatcttttactttcaccagcgtttctgggtgagcaaaaacaggaaggcaaaatgccgcaaaaaagggaataagggcgacacggaaatgttgaatactcatactcttcctttttcaatattattgaagcatttatcagggttattgtctcatgagcggatacatatttgaatgtatttagaaaaataaacaaataggggttccgcgcacatttccccgaaaagtgccacctaaattgtaagcgttaatattttgttaaaattcgcgttaaatttttgttaaatcagctcattttttaaccaataggccgaaatcggcaaaatcccttataaatcaaaagaatagaccgagatagggttgagtgttgttccagtttggaacaagagtccactattaaagaacgtggactccaacgtcaaagggcgaaaaaccgtctatcagggcgatggcccactacgtgaaccatcaccctaatcaagttttttggggtcgaggtgccgtaaagcactaaatcggaaccctaaagggagcccccgatttagagcttgacggggaaagccggcgaacgtggcgagaaaggaagggaagaaagcgaaaggagcgggcgctagggcgctggcaagtgtagcggtcacgctgcgcgtaaccaccacacccgccgcgcttaatgcgccgctacagggcgcgtcccattcgccattcaggctgcgcaactgttgggaagggcgatcggtgcgggcctcttcgctattacgccagctggcgaaagggggatgtgctgcaaggcgattaagttgggtaacgccagggttttcccagtcacgacgttgttttatcggtctgtatatcgaggtttatttattaatttgaatagatattaagttttattatatttacacttacatactaataataaattcaacaaacaatttatttatgtttatttatttattaaaaaaaaacaaaaactcaaaatttcttctataaagtaacaaaacttttatcgaattcctgcagcccgggggatccactagttctagagggacagcccccccccaaagcccccagggatgtaattacgtccctcccccgctagggggcagcagcgagccgcccggggctccgctccggtccggcgctccccccgcatccccgagccggcagcgtgcggggacagcccgggcacggggaaggtggcacgggatcgctttcctctgaacgcttctcgctgctctttgagcctgcagacacctggggggatacggggaaaaggcctccaaggccagcttcccacaataagttgggtgaattttggctcattcctcctttctataggattgaggtcagagctttgtgatgggaattctgtggaatgtgtgtcagttagggtgtggaaagtcccgacattgattattgactagttattaatagtaatcaattacggggtcattagttcatagcccatatatggagttccgcgttacataacttacggtaaatggcccgcctggctgaccgcccaacgacccccgcccattgacgtcaataatgacgtatgttcccatagtaacgccaatagggactttccattgacgtcaatgggtggagtatttacggtaaactgcccacttggcagtacatcaagtgtatcatatgccaagtacgccccctattgacgtcaatgacggtaaatggcccgcctggcattatgcccagtacatgaccttatgggactttcctacttggcagtacatctacgtattagtcatcgctattaccatggtgatgcggttttggcagtacatcaatgggcgtggatagcggtttgactcacggggatttccaagtctccaccccattgacgtcaatgggagtttgttttggcaccaaaatcaacgggactttccaaaatgtcgtaacaactccgccccattgacgcaaatgggcggtaggcgtgtacggtgggaggtctatataagcagagctggtttagtgaaccgtcagatcagatctttgtcgatcctaccatccactcgacacacccgccagcggccgcagttgcgcagccatcgacgtcagacgcggaagcttcgatcaactacgcagacaggtaccaaaacaaatgttctcgtcacgtgggcatgaatctgatgctgtttccctgcagacaatgcgagagaatgaatcagaattcaaatatctgcttcactcacggacagaaagactgtttagagtgctttcccgtgtcagaatctcaacccgtttctgtcgtcaaaaaggcgtatcagaaactgtgctacattcatcatatcatgggaaaggtgccagacgcttgcactgcctgcgatctggtcaatgtggatttggatgactgcatctttgaacaataaatgatttaaatcaggtatgtcttttgttgatcaccctccagattggttggaagaagttggtgaaggtcttcgcgagtttttgggccttgaagcgggcccaccgaaaccaaaacccaatcagcagcatcaagatcaagcccgtggtcttgtgctgcctggttataactatctcggacccggaaacggtctcgatcgaggagagcctgtcaacagggcagacgaggtcgcgcgagagcacgacatctcgtacaacgagcagcttgaggcgggagacaacccctacctcaagtacaaccacgcggacgccgagtttcaggagaagctcgccgacgacacatccttcgggggaaacctcggaaaggcagtctttcaggccaagaaaagggttctcgaaccttttggcctggttgaagagggtgctaagacggcccctaccggaaagcggatagacgaccactttccaaaaagaaagaaggctcggaccgaagaggactccaagccttccacctcgtcagacgccgaagctggacccagcggatcccagcagctgcaaatcccagcccaaccagcctcaagtttgggagctgatacaatgtctgcgggaggtggcggcccattgggcgacaataaccaaggtgccgatggagtgggcaatgcctcgggagattggcattgcgattccacgtggatgggggacagagtcgtcaccaagtccacccgaacctgggtgctgcccagctacaacaaccaccagtaccgagagatcaaaagcggctccgtcgacggaagcaacgccaacgcctactttggatacagcaccccctgggggtactttgactttaaccgcttccacagccactggagcccccgagactggcaaagactcatcaacaactactggggcttcagaccccggtccctcagagtcaaaatcttcaacattcaagtcaaagaggtcacggtgcaggactccaccaccaccatcgccaacaacctcacctccaccgtccaagtgtttacggacgacgactaccagctgccctacgtcgtcggcaacgggaccgagggatgcctgccggccttccctccgcaggtctttacgctgccgcagtacggttacgcgacgctgaaccgcgacaacacagaaaatcccaccgagaggagcagcttcttctgcctagagtactttcccagcaagatgctgagaacgggcaacaactttgagtttacctacaactttgaggaggtgcccttccactccagcttcgctcccagtcagaacctgttcaagctggccaacccgctggtggaccagtacttgtaccgcttcgtgagcacaaataacactggcggagtccagttcaacaagaacctggccgggagatacgccaacacctacaaaaactggttcccggggcccatgggccgaacccagggctggaacctgggctccggggtcaaccgcgccagtgtcagcgccttcgccacgaccaataggatggagctcgagggcgcgagttaccaggtgcccccgcagccgaacggcatgaccaacaacctccagggcagcaacacctatgccctggagaacactatgatcttcaacagccagccggcgaacccgggcaccaccgccacgtacctcgagggcaacatgctcatcaccagcgagagcgagacgcagccggtgaaccgcgtggcgtacaacgtcggcgggcagatggccaccaacaaccagagctccaccactgcccccgcgaccggcacgtacaacctccaggaaatcgtgcccggcagcgtgtggatggagagggacgtgtacctccaaggacccatctgggccaagatcccagagacgggggcgcactttcacccctctccggccatgggcggattcggactcaaacacccaccgcccatgatgctcatcaagaacacgcctgtgcccggaaatatcaccagcttctcggacgtgcccgtcagcagcttcatcacccagtacagcaccgggcaggtcaccgtggagatggagtgggagctcaagaaggaaaactccaagaggtggaacccagagatccagtacacaaacaactacaacgacccccagtttgtggactttgccccggacagcaccggggaatacagaaccaccagacctatcggaacccgataccttacccgacccctttaacccgggagttctagggatctggcggccgctcgagtctagagggcccgtttaaacccgctgatcagcctcgactgtgccttctagttgccagccatctgttgtttgcccctcccccgtgccttccttgaccctggaaggtgccactcccactgtcctttcctaataaaatgaggaaattgcatcgcattgtctgagtaggtgtcattctattctggggggtggggtggggcaggacagcaagggggaggattgggaagacaatagcaggcatgctggggatgcggtgggctctatgggcgatcgctagcgtttaaacttaagcttggtaccgagctcggatccactagtccagtgtggtggaattcctgcttcgcgatgtacgggccagatatacgcgttgtttactcatgtctgggggtgggcgaagaactccagcatgagatccccgcgctggaggatcatccagccggcgtcccggaaaacgattccgaagcccaacctttgcctgcaggtcgactctagaggatccgaaaaaacctcccacacctccccctgaacctgaaacataaaatgaatgcaattgttgttgttaacttgtttattgcagcttataatggttacaaataaagcaatagcatcacaaatttcacaaataaagcatttttttcactgcattctagttgtggtttgtccaaactcatcaatgtatcttatcatgtctggatccccgcggccgcggtacccacgtgggcgcgccatttaaatgataactcagagagagtgtcctcgagccaatctggaagataaccatcggcagccatacctgatttaaatcatttattgttcaaagatgcagtcatccaaatccacattgaccagatcgcaggcagtgcaagcgtctggcacctttcccatgatatgatgaatgtagcacagtttctgatacgcctttttgacgacagaaacgggttgagattctgacacgggaaagcactctaaacagtctttctgtccgtgagtgaagcagatatttgaattctgattcattctctcgcattgtctgcagggaaacagcatcagattcatgcccacgtgacgagaacatttgttttggtacctgtctgcgtagttgatcgaagcttccgcgtctgacgtcgatggctgcgcaactgactcgcgcacccgtttgggctcacttatatctgcgtcactgggggcgggtcttttcttggctccaccctttttgacgtagaattcatgctccacctcaaccacgtgatcctttgcccaccggaaaaagtctttgacttcctgcttggtgaccttcccaaagtcatgatccagacggcgggtgagttcaaatttgaacatccggtcttgcaacggctgctggtgttcgaaggtcgttgagttcccgtcaatcacggcgcacatgttggtgttggaggtgacgatcacgggagtcgggtctatctgggccgaggacttgcatttctggtccacgcgcaccttgcttcctccgagaatggctttggccgactccacgaccttggcggtcatcttcccctcctcccaccagatcaccatcttgtcgacacagtcgttgaagggaaagttctcattggtccagtttacgcacccgtagaagggcacagtgtgggctatggcctccgcgatgttggtcttcccggtagttgcaggcccaaacagccagatggtgttcctcttgccgaactttttcgtggcccatcccagaaagacggaagccgcatattggggatcgtacccgtttagttccaaaattttataaatccgattgctggaaatgtcctccacgggctgctggcccaccaggtagtcgggggcggttttagtcaggctcataatctttcccgcattgtccaaggcagccttgatttgggaccgcgagttggaggccgcattgaaggagatgtatgaggcctggtcctcctggatccactgcttctccgaggtaatccccttgtccacgagccacccgaccagctccatgtacctggctgaagtttttgatctgatcaccggcgcatcagaattgggattctgattctctttgttctgctcctgcgtctgcgacacgtgcgtcagatgctgcgccaccaaccgtttacgctccgtgagattcaaacaggcgcttaaatactgttccatattagtccacgcccactggagctcaggctgggttttggggagcaagtaattggggatgtagcactcatccaccaccttgttcccgcctccggcgccatttctggtctttgtgaccgcgaaccagtttggcaaagtcggctcgatcccgcggtaaattctctgaatcagtttttcgcgaatctgactcaggaaacgtcccaaaaccatggatttcaccccggtggtttccacgagcacgtgcatgtggaagtagctctctcccttctcaaattgcacaaagaaaagggcctccggggccttactcacacggcgccattccgtcagaaagtcgcgctgcagcttctcggccacggtcaggggtgcctgctcaatcagattcagatccatgtcagaatctggcggcaactcccattccttctcggccacccagttcacaaagctgtcagaaatgccgggcagatgctcgtcaaggtcgctggggaccttaatcacaatctcgtaaaaccccggcatggcggcgataactattatcatcgtgtttttcaaaggaaaaccacgtccccgtggttcggggggcctagacgtttttttaacctcgactaaacacatgtaaagcatgtgcaccgaggccccagatcagatcccatacaatggggtaccttctgggcatccttcagccccttgttgaatacgcttgaggagagccatttgactctttccacaactatccaactcacaacgtggcactggggttgtgccgcctttgcaggtgtatcttatacacgtggcttttggccgcagaggcacctgtcgccaggtggggggttccgctgcctgcaaagggtcgctacagacgttgtttgtcttcaagaagcttccagaggaactgcttccttcacgacattcaacagaccttgcattcctttggcgagaggggaaagacccctaggaatgctcgtcaagaagacagggccaggtttccgggccctcacattgccaaaagacggcaatatggtggaaaataacatatagacaaacgcacaccggccttattccaagcggcttcggccagtaacgttagggggggggggcggaattctatccctcagttatctcagagagagtgtcctcgagccaatctggaagataaccatcggcagccatacctgatttaaatcatttattgttcaaagatgcagtcatccaaatccacattgaccagatcgcaggcagtgcaagcgtctggcacctttcccatgatatgatgaatgtagcacagtttctgatacgcctttttgacgacagaaacgggttgagattctgacacgggaaagcactctaaacagtctttctgtccgtgagtgaagcagatatttgaattctgattcattctctcgcattgtctgcagggaaacagcatcagattcatgcccacgtgacgagaacatttgttttggtacctgtctgcgtagttgatcgaagcttccgcgtctgacgtcgatggctgcgcaactgactcgcgcacccgtttgggctcacttatatctgcgtcactgggggcgggtcttttcttggctccaccctttttgacgtagaattcatgctccacctcaaccacgtgatcctttgcccaccggaaaaagtctttgacttcctgcttggtgaccttcccaaagtcatgatccagacggcgggtgagttcaaatttgaacatccggtcttgcaacggctgctggtgttcgaaggtcgttgagttcccgtcaatcacggcgcacatgttggtgttggaggtgacgatcacgggagtcgggtctatctgggccgaggacttgcatttctggtccacgcgcaccttgcttcctccgagaatggctttggccgactccacgaccttggcggtcatcttcccctcctcccaccagatcaccatcttgtcgacacagtcgttgaagggaaagttctcattggtccagtttacgcacccgtagaagggcacagtgtgggctatggcctccgcgatgttggtcttcccggtagttgcaggcccaaacagccagatggtgttcctcttgccgaactttttcgtggcccatcccagaaagacggaagccgcatattggggatcgtacccgtttagttccaaaattttataaatccgattgctggaaatgtcctccacgggctgctggcccaccaggtagtcgggggcggttttagtcaggctcataatctttcccgcattgtccaaggcagccttgatttgggaccgcgagttggaggccgcattgaaggagatgtatgaggcctggtcctcctggatccactgcttctccgaggtaatccccttgtccacgagccacccgaccagctccatggtggcttcggggccgcggaggctggatcggtcccggtgtcttctatggaggtcaaaacagcgtggatggcgtctccaggcgatctgacggttcactaaacgagctctgcttatatagacctcccaccgtacacgcctaccgcccatttgcgtcaatggggcggagttgttacgacattttggaaagtcccgttgattttggtgccaaaacaaactcccattgacgtcaatggggtggagacttggaaatccccgtgagtcaaaccgctatccacgcccattgatgtactgccaaaaccgcatcaccatggtaatagcgatgactaatacgtagatgtactgccaagtaggaaagtcccataaggtcatgtactgggcataatgccaggcgggccatttaccgtcattgacgtcaatagggggcgtacttggcatatgatacacttgatgtactgccaagtgggcagtttaccgtaaatactccacccattgacgtcaatggaaagtccctattggcgttactatgggaacatacgtcattattgacgtcaatgggcgggggtcgttgggcggtcagccaggcgggccatttaccgtaagttatgtaacgcggaactccatatatgggctatgaactaatgaccccgtaattgattactattaataactagtcaataatcaatgtcttacatccctgggggctttgggggggggctgtccctctagagcggccgccaccgcggtggagctccagcttttgttccctttagtgagggttaattagatcttaatacgactcactatagggcgaattgggtaccgggccccccctcgaggtcgacggtatcgtgtgaaattgttatccgctcacaattccacacaacatacgagccggaagcataaagtgtaaagcctggggtgcctaatgagtgagctaactcacattaattgcgttgcgctcactgcccgctttccagtcgggaaacctgtcgtgccagctgcattaatgaatcggccaacgcgcggggagaggcggtttgcgtattgggcgctcttccgcttcctcgctcactgactcgctgcgctcggtcgttcggctgcggcgagcggtatcagctcactcaaaggcggtaatacggttatccacagaatcaggggataacgcaggaaagaacatgtgagcaaaaggccagcaaaaggccaggaaccgtaaaaaggccgcgttgctggcgtt

SEQ ID NO: 3 - DNA, 11635 bp, synthetic construct
  misc_feature 1..11635: note = plasmid
  source 1..11635: mol_type = other DNA
ggtacccaactccatgcttaacagtccccaggtacagcccaccctgcgtcgcaaccaggaacagctctacagcttcctggagcgccactcgccctacttccgcagccacagtgcgcagattaggagcgccacttctttttgtcacttgaaaaacatgtaaaaataatgtactaggagacactttcaataaaggcaaatgtttttatttgtacactctcgggtgattatttaccccccacccttgccgtctgcgccgtttaaaaatcaaaggggttctgccgcgcatcgctatgcgccactggcagggacacgttgcgatactggtgtttagtgctccacttaaactcaggcacaaccatccgcggcagctcggtgaagttttcactccacaggctgcgcaccatcaccaacgcgtttagcaggtcgggcgccgatatcttgaagtcgcagttggggcctccgccctgcgcgcgcgagttgcgatacacagggttgcagcactggaacactatcagcgccgggtggtgcacgctggccagcacgctcttgtcggagatcagatccgcgtccaggtcctccgcgttgctcagggcgaacggagtcaactttggtagctgccttcccaaaaagggtgcatgcccaggctttgagttgcactcgcaccgtagtggcatcagaaggtgaccgtgcccggtctgggcgttaggatacagcgcctgcatgaaagccttgatctgcttaaaagccacctgagcctttgcgccttcagagaagaacatgccgcaagacttgccggaaaactgattggccggacaggccgcgtcatgcacgcagcaccttgcgtcggtgttggagatctgcaccacatttcggccccaccggttcttcacgatcttggccttgctagactgctccttcagcgcgcgctgcccgttttcgctcgtcacatccatttcaatcacgtgctccttatttatcataatgctcccgtgtagacacttaagctcgccttcgatctcagcgcagcggtgcagccacaacgcgcagcccgtgggctcgtggtgcttgtaggttacctctgcaaacgactgcaggtacgcctgcaggaatcgccccatcatcgtcacaaaggtcttgttgctggtgaaggtcagctgcaacccgcggtgctcctcgtttagccaggtcttgcatacggccgccagagcttccacttggtcaggcagtagcttgaagtttgcctttagatcgttatccacgtggtacttgtccatcaacgcgcgcgcagcctccatgcccttctcccacgcagacacgatcggcaggctcagcgggtttatcaccgtgctttcactttccgcttcactggactcttccttttcctcttgcgtccgcataccccgcgccactgggtcgtcttcattcagccgccgcaccgtgcgcttacctcccttgccgtgcttgattagcaccggtgggttgctgaaacccaccatttgtagcgccacatcttctctttcttcctcgctgtccacgatcacctctggggatggcgggcgctcgggcttgggagaggggcgcttctttttctttttggacgcaatggccaaatccgccgtcgaggtcgatggccgcgggctgggtgtgcgcggcaccagcgcatcttgtgacgagtcttcttcgtcctcggactcgagacgccgcctcagccgcttttttgggggcgcgcggggaggcggcggcgacggcgacggggacgacacgtcctccatggttggtggacgtcgcgccgcaccgcgtccgcgctcgggggtggtttcgcgctgctcctcttcccgactggccatttccttctcctataggcagaaaaagatcatggagtcagtcgagaaggaggacagcctaaccgccccctttgagttcgccaccaccgcctccaccgatgccgccaacgcgcctaccaccttccccgtcgaggcacccccgcttgaggaggaggaagtgattatcgagcaggacccaggttttgtaagcgaagacgacgaggatcgctcagtaccaacagaggataaaaagcaagaccaggacgacgcagaggcaaacgaggaacaagtcgggcggggggaccaaaggcatggcgactacctagatgtgggagacgacgtgctgttgaagcatctgcagcgccagtgcgccattatctgcgacgcgttgcaagagcgcagcgatgtgcccctcgccatagcggatgtcagccttgcctacgaacgccacctgttctcaccgcgcgtaccccccaaacgccaagaaaacggcacatgcgagcccaacccgcgcctcaacttctaccccgtatttgccgtgccagaggtgcttgccacctatcacatctttttccaaaactgcaagatacccctatcctgccgtgccaaccgcagccgagcggacaagcagctggccttgcggcagggcgctgtcatacctgatatcgcctcgctcgacgaagtgccaaaaatctttgagggtcttggacgcgacgagaaacgcgcggcaaacgctctgcaacaagaaaacagcgaaaatgaaagtcactgtggagtgctggtggaacttgagggtgacaacgcgcgcctagccgtgctgaaacgcagcatcgaggtcacccactttgcctacccggcacttaacctaccccccaaggttatgagcacagtcatgagcgagctgatcgtgcgccgtgcacgacccctggagagggatgcaaacttgcaagaacaaaccgaggagggcctacccgcagttggcgatgagcagctggcgcgctggcttgagacgcgcgagcctgccgacttggaggagcgacgcaagctaatgatggccgcagtgcttgttaccgtggagcttgagtgcatgcagcggttctttgctgacccggagatgcagcgcaagctagaggaaacgttgcactacacctttcgccagggctacgtgcgccaggcctgcaaaatttccaacgtggagctctgcaacctggtctcctaccttggaattttgcacgaaaaccgcctcgggcaaaacgtgcttcattccacgctcaagggcgaggcgcgccgcgactacgtccgcgactgcgtttacttatttctgtgctacacctggcaaacggccatgggcgtgtggcagcaatgcctggaggagcgcaacctaaaggagctgcagaagctgctaaagcaaaacttgaaggacctatggacggccttcaacgagcgctccgtggccgcgcacctggcggacattatcttccccgaacgcctgcttaaaaccctgcaacagggtctgccagacttcaccagtcaaagcatgttgcaaaactttaggaactttatcctagagcgttcaggaattctgcccgccacctgctgtgcgcttcctagcgactttgtgcccattaagtaccgtgaatgccctccgccgctttggggtcactgctaccttctgcagctagccaactaccttgcctaccactccgacatcatggaagacgtgagcggtgacggcctactggagtgtcactgtcgctgcaacctatgcaccccgcaccgctccctggtctgcaattcgcaactgcttagcgaaagtcaaattatcggtacctttgagctgcagggtccctcgcctgacgaaaagtccgcggctccggggttgaaactcactccggggctgtggacgtcggcttaccttcgcaaatttgtacctgaggactaccacgcccacgagattaggttctacgaagaccaatcccgcccgccaaatgcggagcttaccgcctgcgtcattacccagggccacatccttggccaattgcaagccatcaacaaagcccgccaagagtttctgctacgaaagggacggggggtttacctggacccccagtccggcgaggagctcaacccaatccccccgccgccgcagccctatcagcagccgcgggcccttgcttcccaggatggcacccaaaaagaagctgcagctgccgccgccgccacccacggacgaggaggaatactgggacagtcaggcagaggaggttttggacgaggaggaggagatgatggaagactgggacagcctagacgaagcttccgaggccgaagaggtgtcagacgaaacaccgtcaccctcggtcgcattcccctcgccggcgccccagaaattggcaaccgttcccagcatcgctacaacctccgctcctcaggcgccgccggcactgcctgttcgccgacccaaccgtagatgggacaccactggaaccagggccggtaagtctaagcagccgccgccgttagcccaagagcaacaacagcgccaaggctaccgctcgtggcgcgggcacaagaacgccatagttgcttgcttgcaagactgtgggggcaacatctccttcgcccgccgctttcttctctaccatcacggcgtggccttcccccgtaacatcctgcattactaccgtcatctctacagcccctactgcaccggcggcagcggcagcggcagcaacagcagcggtcacacagaagcaaaggcgaccggatagcaagactctgacaaagcccaagaaatccacagcggcggcagcagcaggaggaggagcgctgcgtctggcgcccaacgaacccgtatcgacccgcgagcttagaaataggatttttcccactctgtatgctatatttcaacaaagcaggggccaagaacaagagctgaaaataaaaaacaggtctctgcgctccctcacccgcagctgcctgtatcacaaaagcgaagatcagcttcggcgcacgctggaagacgcggaggctctcttcagcaaatactgcgcgctgactcttaaggactagtttcgcgccctttctcaaatttaagcgcgaaaactacgtcatctccagcggccacacccggcgccagcacctgtcgtcagcgccattatgagcaaggaaattcccacgccctacatgtggagttaccagccacaaatgggacttgcggctggagctgcccaagactactcaacccgaataaactacatgagcgcgggaccccacatgatatcccgggtcaacggaatccgcgcccaccgaaaccgaattctcctcgaacaggcggctattaccaccacacctcgtaataaccttaatccccgtagttggcccgctgccctggtgtaccaggaaagtcccgctcccaccactgtggtacttcccagagacgcccaggccgaagttcagatgactaactcaggggcgcagcttgcgggcggctttcgtcacagggtgcggtcgcccgggcgttttagggcggagtaacttgcatgtattgggaattgtagtttttttaaaatgggaagtgacgtatcgtgggaaaacggaagtgaagatttgaggaagttgtgggttttttggctttcgtttctgggcgtaggttcgcgtgcggttttctgggtgttttttgtggactttaaccgttacgtcattttttagtcctatatatactcgctctgtacttggccctttttacactgtgactgattgagctggtgccgtgtcgagtggtgttttttaataggtttttttactggtaaggctgactgttatggctgccgctgtggaagcgctgtatgttgttctggagcgggagggtgctattttgcctaggcaggagggtttttcaggtgtttatgtgtttttctctcctattaattttgttatacctcctatgggggctgtaatgttgtctctacgcctgcgggtatgtattcccccgggctatttcggtcgctttttagcactgaccgatgttaaccaacctgatgtgtttaccgagtcttacattatgactccggacatgaccgaggaactgtcggtggtgctttttaatcacggtgaccagtttttttacggtcacgccggcatggccgtagtccgtcttatgcttataagggttgtttttcctgttgtaagacaggcttctaatgtttaaatgtttttttttttgttattttattttgtgtttaatgcaggaacccgcagacatgtttgagagaaaaatggtgtctttttctgtggtggttccggaacttacctgcctttatctgcatgagcatgactacgatgtgcttgcttttttgcgcgaggctttgcctgattttttgagcagcaccttgcattttatatcgccgcccatgcaacaagcttacataggggctacgctggttagcatagctccgagtatgcgtgtcataatcagtgtgggttcttttgtcatggttcctggcggggaagtggccgcgctggtccgtgcagacctgcacgattatgttcagctggccctgcgaagggacctacgggatcgcggtatttttgttaatgttccgcttttgaatcttatacaggtctgtgaggaacctgaatttttgcaatcatgattcgctgcttgaggctgaaggtggagggcgctctggagcagatttttacaatggccggacttaatattcgggatttgcttagagacatattgataaggtggcgagatgaaaattatttgggcatggttgaaggtgctggaatgtttatagaggagattcaccctgaagggtttagcctttacgtccacttggacgtgagggcagtttgccttttggaagccattgtgcaacatcttacaaatgccattatctgttctttggctgtagagtttgaccacgccaccggaggggagcgcgttcacttaatagatcttcattttgaggttttggataatcttttggaataaaaaaaaaaaaacatggttcttccagctcttcccgctcctcccgtgtgtgactcgcagaacgaatgtgtaggttggctgggtgtggcttattctgcggtggtggatgttatcagggcagcggcgcatgaaggagtttacatagaacccgaagccagggggcgcctggatgctttgagagagtggatatactacaactactacacagagcgagctaagcgacgagaccggagacgcagatctgtttgtcacgcccgcacctggttttgcttcaggaaatatgactacgtccggcgttccatttggcatgacactacgaccaacacgatctcggttgtctcggcgcactccgtacagtagggatcgcctacctccttttgagacagagacccgcgctaccatactggaggatcatccgctgctgcccgaatgtaacactttgacaatgcacaacgtgagttacgtgcgaggtcttccctgcagtgtgggatttacgctgattcaggaatgggttgttccctgggatatggttctgacgcgggaggagcttgtaatcctgaggaagtgtatgcacgtgtgcctgtgttgtgccaacattgatatcatgacgagcatgatgatccatggttacgagtcctgggctctccactgtcattgttccagtcccggttccctgcagtgcatagccggcgggcaggttttggccagctggtttaggatggtggtggatggcgccatgtttaatcagaggtttatatggtaccgggaggtggtgaattacaacatgccaaaagaggtaatgtttatgtccagcgtgtttatgaggggtcgccacttaatctacctgcgcttgtggtatgatggccacgtgggttctgtggtccccgccatgagctttggatacagcgccttgcactgtgggattttgaacaatattgtggtgctgtgctgcagttactgtgctgatttaagtgagatcagggtgcgctgctgtgcccggaggacaaggcgtctcatgctgcgggcggtgcgaatcatcgctgaggagaccactgccatgttgtattcctgcaggacggagcggcggcggcagcagtttattcgcgcgctgctgcagcaccaccgccctatcctgatgcacgattatgactctacccccatgtaggcgtggacttccccttcgccgcccgttgagcaaccgcaagttggacagcagcctgtggctcagcagctggacagcgacatgaacttaagcgagctgcccggggagtttattaatatcactgatgagcgtttggctcgacaggaaaccgtgtggaatataacacctaagaatatgtctgttacccatgatatgatgctttttaaggccagccggggagaaaggactgtgtactctgtgtgttgggagggaggtggcaggttgaatactagggttctgtgagtttgattaaggtacggtgatcaatataagctatgtggtggtggggctatactactgaatgaaaaatgacttgaaattttctgcaattgaaaaataaacacgttgaaacataacatgcaacaggttcacgattctttattcctgggcaatgtaggagaaggtgtaagagttggtagcaaaagtttcagtggtgtattttccactttcccaggaccatgtaaaagacatagagtaagtgcttacctcgctagtttctgtggattcactagaatcgatgtaggatgttgcccctcctgacgcggtaggagaaggggagggtgccctgcatgtctgccgctgctcttgctcttgccgctgctgaggaggggggcgcatctgccgcagcaccggatgcatctgggaaaagcaaaaaaggggctcgtccctgtttccggaggaatttgcaagcggggtcttgcatgacggggaggcaaacccccgttcgccgcagtccggccggcccgagactcgaaccgggggtcctgcgactcaacccttggaaaataaccctccggctacagggagcgagccacttaatgctttcgctttccagcctaaccgcttacgccgcgcgcggccagtggccaaaaaagctagcgcagcagccgccgcgcctggaaggaagccaaaaggagcgctcccccgttgtctgacgtcgcacacctgggttcgacacgcgggcggtaaccgcatggatcacggcggacggccggatccggggttcgaaccccggtcgtccgccatgatacccttgcgaatttatccaccagaccacggaagagtgcccgcttacaggctctccttttgcacggtctagagcgtcaacgactgcgcacgcctcaccggccagagcgtcccgaccatggagcactttttgccgctgcgcaacatctggaaccgcgtccgcgactttccgcgcgcctccaccaccgccgccggcatcacctggatgtccaggtacatctacggattacgtcgacgtttaaaccatatgatcagctcactcaaaggcggtaatacggttatccacagaatcaggggataacgcaggaaagaacatgtgagcaaaaggccagcaaaaggccaggaaccgtaaaaaggccgcgttgctggcgtttttccataggctccgcccccctgacgagcatcacaaaaatcgacgctcaagtcagaggtggcgaaacccgacaggactataaagataccaggcgtttccccctggaagctccctcgtgcgctctcctgttccgaccctgccgcttaccggatacctgtccgcctttctcccttcgggaagcgtggcgctttctcatagctcacgctgtaggtatctcagttcggtgtaggtcgttcgctccaagctgggctgtgtgcacgaaccccccgttcagcccgaccgctgcgccttatccggtaactatcgtcttgagtccaacccggtaagacacgacttatcgccactggcagcagccactggtaacaggattagcagagcgaggtatgtaggcggtgctacagagttcttgaagtggtggcctaactacggctacactagaagaacagtatttggtatctgcgctctgctgaagccagttaccttcggaaaaagagttggtagctcttgatccggcaaacaaaccaccgctggtagcggtggtttttttgtttgcaagcagcagattacgcgcagaaaaaaaggatctcaagaagatcctttgatcttttctacggggtctgacgctcagtggaacgaaaactcacgttaagggattttggtcatgagattatcaaaaaggatcttcacctagatccttttaaattaaaaatgaagttttaaatcaatctaaagtatatatgagtaaacttggtctgacagttaccaatgcttaatcagtgaggcacctatctcagcgatctgtctatttcgttcatccatagttgcctgactccccgtcgtgtagataactacgatacgggagggcttaccatctggccccagtgctgcaatgataccgcgagacccacgctcaccggctccagatttatcagcaataaaccagccagccggaagggccgagcgcagaagtggtcctgcaactttatccgcctccatccagtctattaattgttgccgggaagctagagtaagtagttcgccagttaatagtttgcgcaacgttgttgccattgctacaggcatcgtggtgtcacgctcgtcgtttggtatggcttcattcagctccggttcccaacgatcaaggcgagttacatgatcccccatgttgtgcaaaaaagcggttagctccttcggtcctccgatcgttgtcagaagtaagttggccgcagtgttatcactcatggttatggcagcactgcataattctcttactgtcatgccatccgtaagatgcttttctgtgactggtgagtactcaaccaagtcattctgagaatagtgtatgcggcgaccgagttgctcttgcccggcgtcaatacgggataataccgcgccacatagcagaactttaaaagtgctcatcattggaaaacgttcttcggggcgaaaactctcaaggatcttaccgctgttgagatccagttcgatgtaacccactcgtgcacccaactgatcttcagcatcttttactttcaccagcgtttctgggtgagcaaaaacaggaaggcaaaatgccgcaaaaaagggaataagggcgacacggaaatgttgaatactcatactcttcctttttcaatattattgaagcatttatcagggttattgtctcatgagcggatacatatttgaatgtatttagaaaaataaacaaataggggttccgcgcacatttccccgaaaagtgccacctaaattgtaagcgttaatattttgttaaaattcgcgttaaatttttgttaaatcagctcattttttaaccaataggccgaaatcggcaaaatcccttataaatcaaaagaatagaccgagatagggttgagtgttgttccagtttggaacaagagtccactattaaagaacgtggactccaacgtcaaagggcgaaaaaccgtctatcagggcgatggcccactacgtgaaccatcaccctaatcaagttttttggggtcgaggtgccgtaaagcactaaatcggaaccctaaagggagcccccgatttagagcttgacggggaaagccggcgaacgtggcgagaaaggaagggaagaaagcgaaaggagcgggcgctagggcgctggcaagtgtagcggtcacgctgcgcgtaaccaccacacccgccgcgcttaatgcgccgctacagggcgcgatggatcc